European Patent Application EP 4 696 783 A1, published February 18, 2026. Title: Filtration speed improvement method. Applicant: KAO CORPORATION. The sequence listing filed with the application follows.

SEQUENCE LISTING (31 sequences)

SEQ ID NO: 1 - DNA, 915 bp, Bacillus subtilis
  source 1..915: mol_type = genomic DNA
atgagaattaaccacaatattgcagcgcttaacacactgaaccgtttgtcttcaaacaacagtgcgagccaaaagaacatggagaaactttcttcaggtcttcgcatcaaccgtgcgggagatgacgcagcaggtcttgcgatctctgaaaaaatgagaggacaaatcagaggtcttgaaatggcttctaaaaactctcaagacggaatctctcttatccaaacagctgagggtgcattaactgaaactcatgcgatccttcaacgtgttcgtgagctagttgttcaagctggaaacactggaactcaggacaaagcaactgatttgcaatctattcaagatgaaatttcagctttaacagatgaaatcgatggtatttcaaatcgtacagaattcaatggtaagaaattgctcgatggcacttacaaagttgacacagctactcctgcaaatcaaaagaacttggtattccaaatcggagcaaatgctacacagcaaatctctgtaaatattgaggatatgggtgctgacgctcttggaattaaagaagctgatggttcaattgcagctcttcattcagttaatgatcttgacgtaacaaaattcgcagataatgcagcagatactgctgatatcggtttcgatgctcaattgaaagttgttgatgaagcgatcaaccaagtttcttctcaacgtgctaagcttggtgcggtacaaaatcgtctagagcacacaattaacaacttaagcgcttctggtgaaaacttgacagctgctgagtctcgtatccgtgacgttgacatggctaaagagatgagcgaattcacaaagaacaacattctttctcaggcttctcaagctatgcttgctcaagcaaaccaacagccgcaaaacgtacttcaattattacgttaa

SEQ ID NO: 2 - protein, 304 aa, Bacillus subtilis
MRINHNIAALNTLNRLSSNNSASQKNMEKLSSGLRINRAGDDAAGLAISEKMRGQIRGLEMASKNSQDGISLIQTAEGALTETHAILQRVRELVVQAGNTGTQDKATDLQSIQDEISALTDEIDGISNRTEFNGKKLLDGTYKVDTATPANQKNLVFQIGANATQQISVNIEDMGADALGIKEADGSIAALHSVNDLDVTKFADNAADTADIGFDAQLKVVDEAINQVSSQRAKLGAVQNRLEHTINNLSASGENLTAAESRIRDVDMAKEMSEFTKNNILSQASQAMLAQANQQPQNVLQLLR

SEQ ID NO: 3 - DNA, 930 bp, Bacillus licheniformis
  source 1..930: mol_type = genomic DNA
atgagaatcaaccacaacattgcagcgcttaacacgctgaaccgtctgtcagcaaacaacggcgcaagccaaaagaacatggagaagctttcttctggtcttcgcatcaaccgtgccggagatgacgcagcaggtcttgcaatctctgaaaaaatgagaggacaaatccgcggtcttgaaatggcttctaagaacgctcaagacggcatctctcttatccaaacagctgaaggtgcattgactgagactcactcaatccttcaacgtgttcgtgaactagttgttcaagctggaaacactggaacacaacaaactgaggatttaacagctatccaagacgagatcaaagcattaaaagacgaaattgacggcatctcagaacgtacggaattcaacggtaaaaaattgttggatggtactttcaaagcaccagcagatccagcaaacccagctgcaggtgaaaaatctttagttttccaaattggagctaacgcaacacaacaaatttctgttaacattgaaaaaatgagcactgatgcattaggagtcaaagatcctgcagatactacgggcagaactctagtaaccaaccaatcagttaaagatatcgatgtaactaaatttgctgataatgcagcaactgcaacagatgtaggttttgatactcaacttaaaatcgttgattcagcgatcaaccaagtatctgcacaacgtgctaaacttggtgcggtacaaaaccgtctagagcacacaatcaacaaccttggtgcttcttctgaaaacttgacagctgctgagtctcgtatccgcgacgttgacatggctaaagaaatgagcgagttcacaaagaacaacattctttctcaagcttctcaagctatgcttgctcaagcgaaccaacagccgcaaaacgttcttcagttgcttcgt

SEQ ID NO: 4 - protein, 310 aa, Bacillus licheniformis
MRINHNIAALNTLNRLSANNGASQKNMEKLSSGLRINRAGDDAAGLAISEKMRGQIRGLEMASKNAQDGISLIQTAEGALTETHSILQRVRELVVQAGNTGTQQTEDLTAIQDEIKALKDEIDGISERTEFNGKKLLDGTFKAPADPANPAAGEKSLVFQIGANATQQISVNIEKMSTDALGVKDPADTTGRTLVTNQSVKDIDVTKFADNAATATDVGFDTQLKIVDSAINQVSAQRAKLGAVQNRLEHTINNLGASSENLTAAESRIRDVDMAKEMSEFTKNNILSQASQAMLAQANQQPQNVLQLLR

SEQ ID NO: 5 - DNA, 822 bp, Brevibacillus brevis
  source 1..822: mol_type = genomic DNA
atgattatccaacacaatatgtctgctcaaaacactcatcgtcaactgggtgtaaacactggcaacctgtctaaaaacgttgaaaaattgtcttccggctaccgcatcaaccgtgcggctgacgatgctgctggtctctccatctccgagcgtatgcgtgcacaagttcgtggtatggaacaagcttcccgcaactcccaagacggtatctctttgatccaaactgctgaaggtgctttgcaaactgtgaacaacatgctcgttcgtattaaagaactggcaacacaatctgcaaacggaacttacactgatactgaagaccgtgctcgtatccaagaagaagtatctgaactgagcaaagaggttgacaacatcaaagacaacaccaaattcaacggtatttctctgctgaatggtaacggcagcaaaaatatcgatctgcaaattggtcaagaaaaagctcaaacactgactttggatgttactaaattcgaccttacagctgttgcatctgcagtaaaagcatatgctcttggtactcaatctggtgcaaaatctgcactgggcgacgttgaagctcaaatcaacaaagtatctgctgctcgttcttacctgggtgcgaaccaaaaccgtctggaaaacactatcaacaacctgaacatcacttctgagaacctgactgctgctgaatcccgtatccgtgacgttgatatggcgaaagagcaaatggcattcactaagaataacattttgactcaagcgtcccaagcaatgttggcacaagctaaccaattgccacaaggcgtactgcaattgctccgt

SEQ ID NO: 6 - protein, 274 aa, Brevibacillus brevis
MIIQHNMSAQNTHRQLGVNTGNLSKNVEKLSSGYRINRAADDAAGLSISERMRAQVRGMEQASRNSQDGISLIQTAEGALQTVNNMLVRIKELATQSANGTYTDTEDRARIQEEVSELSKEVDNIKDNTKFNGISLLNGNGSKNIDLQIGQEKAQTLTLDVTKFDLTAVASAVKAYALGTQSGAKSALGDVEAQINKVSAARSYLGANQNRLENTINNLNITSENLTAAESRIRDVDMAKEQMAFTKNNILTQASQAMLAQANQLPQGVLQLLR

SEQ ID NO: 7 - DNA, 1494 bp, Escherichia coli fliC
  source 1..1494: mol_type = genomic DNA
atggcacaagtcattaataccaacagcctctcgctgatcactcaaaataatatcaacaagaaccagtctgcgctgtcgagttctatcgagcgtctgtcttctggcttgcgtattaacagcgcgaaggatgacgcagcgggtcaggcgattgctaaccgtttcacctctaacattaaaggcctgactcaggcggcccgtaacgccaacgacggtatctccgttgcgcagaccaccgaaggcgcgctgtccgaaatcaacaacaacttacagcgtgtgcgtgaactgacggtacaggccactaccggtactaactctgagtctgatctgtcttctatccaggacgaaattaaatcccgtctggatgaaattgaccgcgtatctggtcagacccagttcaacggcgtgaacgtgctggcaaaaaatggctccatgaaaatccaggttggcgcaaatgataaccagactatcactatcgatctgaagcagattgatgctaaaactcttggccttgatggttttagcgttaaaaataacgatacagttaccactagtgctccagtaactgcttttggtgctaccaccacaaacaatattaaacttactggaattaccctttctacggaagcagccactgatactggcggaactaacccagcttcaattgagggtgtttatactgataatggtaatgattactatgcgaaaatcaccggtggtgataacgatgggaagtattacgcagtaacagttgctaatgatggtacagtgacaatggcgactggagcaacggcaaatgcaactgtaactgatgcaaatactactaaagctacaactatcacttcaggcggtacacctgttcagattgataatactgcaggttccgcaactgccaaccttggtgctgttagcttagtaaaactgcaggattccaagggtaatgataccgatacatatgcgcttaaagatacaaatggcaatctttacgctgcggatgtgaatgaaactactggtgctgtttctgttaaaactattacctatactgactcttccggtgccgccagttctccaaccgcggtcaaactgggcggagatgatggcaaaacagaagtggtcgatattgatggtaaaacatacgattctgccgatttaaatggcggtaatctgcaaacaggtttgactgctggtggtgaggctctgactgctgttgcaaatggtaaaaccacggatccgctgaaagcgctggacgatgctatcgcatctgtagacaaattccgttcttccctcggtgcggtgcaaaaccgtctggattccgcggttaccaacctgaacaacaccactaccaacctgtctgaagcgcagtcccgtattcaggacgccgactatgcgaccgaagtgtccaatatgtcgaaagcgcagatcatccagcaggccggtaactccgtgttggcaaaagctaaccaggtaccgcagcaggttctgtctctgctgcagggt

SEQ ID NO: 8 - protein, 498 aa, Escherichia coli fliC
MAQVINTNSLSLITQNNINKNQSALSSSIERLSSGLRINSAKDDAAGQAIANRFTSNIKGLTQAARNANDGISVAQTTEGALSEINNNLQRVRELTVQATTGTNSESDLSSIQDEIKSRLDEIDRVSGQTQFNGVNVLAKNGSMKIQVGANDNQTITIDLKQIDAKTLGLDGFSVKNNDTVTTSAPVTAFGATTTNNIKLTGITLSTEAATDTGGTNPASIEGVYTDNGNDYYAKITGGDNDGKYYAVTVANDGTVTMATGATANATVTDANTTKATTITSGGTPVQIDNTAGSATANLGAVSLVKLQDSKGNDTDTYALKDTNGNLYAADVNETTGAVSVKTITYTDSSGAASSPTAVKLGGDDGKTEVVDIDGKTYDSADLNGGNLQTGLTAGGEALTAVANGKTTDPLKALDDAIASVDKFRSSLGAVQNRLDSAVTNLNNTTTNLSEAQSRIQDADYATEVSNMSKAQIIQQAGNSVLAKANQVPQQVLSLLQG

SEQ ID NO: 9 - DNA, 780 bp, Clostridium butyricum flaA
  source 1..780: mol_type = genomic DNA
ttagcgagttgtgatcaattaaagaaaaataataaggataatattagtgctaaaatgaagttgacatctggttatagaataaactatgcggcagatgatgcagcaggtctatgtatatcggaaaaaatgagaactcaaattaaaggccttaatcaagcaagcacgaatactcaagatggatattctatgtttcaaactatagaaagctcaacggaagaagtacacaatattttacaaagaatgtctatattatcaacacagtcggttactgaaactaataccaatgatgatagaaagctggtagacaaggaagtacaacagcttaaagaagaaatagatagaatagctaaagatacagaatttaatggtaaaaaggttttggatggaacatatggaataggtggggaaagattggatattatggttggagaaaatcctggatttataatttcatttccaccaatagatagtgttgaatgcaattctttggggattggagatttaagagtagatacaaaagaagattcccaaaaagctcttaaagcattatcaaaggcaattgatgaaatttcatcaagaagagttgagatgggggctacgggcaatagattaactcatgcagttaagtcactagataataattcagaaaacatgtccgcatcggaatcaagaattagagatactgatattgcaaaagaagcgatggaaaatgttaaaagtaatattttaataaattctactcaatcagtattagcacaatcaaatcatgagccggagtat

SEQ ID NO: 10 - protein, 260 aa, Clostridium butyricum flaA
LASCDQLKKNNKDNISAKMKLTSGYRINYAADDAAGLCISEKMRTQIKGLNQASTNTQDGYSMFQTIESSTEEVHNILQRMSILSTQSVTETNTNDDRKLVDKEVQQLKEEIDRIAKDTEFNGKKVLDGTYGIGGERLDIMVGENPGFIISFPPIDSVECNSLGIGDLRVDTKEDSQKALKALSKAIDEISSRRVEMGATGNRLTHAVKSLDNNSENMSASESRIRDTDIAKEAMENVKSNILINSTQSVLAQSNHEPEY

SEQ ID NO: 11 - DNA, 1072 bp, synthetic construct
  source 1..1072: mol_type = other DNA
taagaaaagtgattctgggagagccgggatcacttttttatttaccttatgcccgaaatgaaagctttatgacctaattgtgtaactatatcctattttttcaaaaaatattttaaaaacgagcaggatttcagaaaaaatcgtggaattgatacactaatgcttttatatagggaaaaggaggtgaactactatgaagaaaatcgcaatagcagctatcactgctacaagcatcctcgctctcagtgcttgcagcagcggcgacaaagaagttatcgcaaaaacagacgcaggcgatgtcacaaaaggcgagctttacacaaacatgaagaaaacagctggcgcaagcgtactgacacagctagtgcaagaaaaagtattggacaagaagtataaagtttcggataaagaaattgacaacaagctgaaagaatacaaaacgcagcttggcgatcaatatactgccctcgaaaagcaatatggcaaagattacctgaaagaacaagtaaaatatgaattgctgacacaaaaagcggctaaagataacatcaaagtaacagacgccgatatcaaagagtactgggaaggcttaaaaggcaaaatccgtgcaagccacatccttgttgctgataaaaagacagctgaagaagtagagaaaaagctgaaaaaaggcgagaagtttgaagaccttgcgaaagaatactcaacagacagctctgcttcaaaaggcggggatcttggctggttcgcaaaagaaggccaaatggacgaaacattcagcaaagctgcattcaaattaaaaacaggtgaagtcagtgatcctgtcaaaacgcaatacggctaccatatcattaaaaagacagaagaacgcggcaaatatgatgatatgaaaaaagaactgaaatctgaagtgcttgaacaaaaattaaatgacaacgcagctgttcaggaagctgttcaaaaagtcatgaagaaggctgacatcgaagtaaaagataaagatctgaaagacacatttaatacatcttcaacaagcaacagcacttcttcatcttcaagcaattctaaataa

SEQ ID NO: 12 - DNA, 28 bp, synthetic construct
  source 1..28: mol_type = other DNA
tttcaaatgagtagaaataatgcacatc

SEQ ID NO: 13 - DNA, 39 bp, synthetic construct
  source 1..39: mol_type = other DNA
tgggtaggatccgcgccgctgtttgtgtgtacaccgcca

SEQ ID NO: 14 - DNA, 43 bp, synthetic construct
  source 1..43: mol_type = other DNA
acacacaaacagcggcgcggatcctacccaatcagtacgttaa

SEQ ID NO: 15 - DNA, 43 bp, synthetic construct; identical to SEQ ID NO: 14
  source 1..43: mol_type = other DNA

SEQ ID NO: 16 - DNA, 20 bp, synthetic construct
  source 1..20: mol_type = other DNA
acacacaaacagcggcgcgg

SEQ ID NO: 17 - DNA, 26 bp, synthetic construct
  source 1..26: mol_type = other DNA
cttttgtttctatcgcttttaattcg

SEQ ID NO: 18 - DNA, 24 bp, synthetic construct
  source 1..24: mol_type = other DNA
gaaatgtgctccccgacaaaattg

SEQ ID NO: 19 - DNA, 23 bp, synthetic construct
  source 1..23: mol_type = other DNA
ttggccgctccgttagaaacagc

SEQ ID NO: 20 - DNA, 28 bp, synthetic construct
  source 1..28: mol_type = other DNA
tttcaaatgagtagaaataatgcacatc

SEQ ID NO: 21 - DNA, 22 bp, synthetic construct
  source 1..22: mol_type = other DNA
ttccaggctgcttcaactttag

SEQ ID NO: 22 - DNA, 30 bp, synthetic construct
  source 1..30: mol_type = other DNA
tcattcatacgaagtaccatggccaaatga

SEQ ID NO: 23 - DNA, 40 bp, synthetic construct
  source 1..40: mol_type = other DNA
cgccaaggtcttttttaaaatgttttgttcctccctgaat

SEQ ID NO: 24 - DNA, 40 bp, synthetic construct
  source 1..40: mol_type = other DNA
attcagggaggaacaaaacattttaaaaaagaccttggcg

SEQ ID NO: 25 - DNA, 40 bp, synthetic construct
  source 1..40: mol_type = other DNA
ctgattgggtaggatccgcgcagttttgctctgatacgtg

SEQ ID NO: 26 - DNA, 24 bp, synthetic construct
  source 1..24: mol_type = other DNA
cgcggatcctacccaatcagtacg

SEQ ID NO: 27 - DNA, 22 bp, synthetic construct
  source 1..22: mol_type = other DNA
cgacagcggaattgactcaagc

SEQ ID NO: 28 - DNA, 38 bp, synthetic construct
  source 1..38: mol_type = other DNA
gagtcaattccgctgtcgtcttcaggtcttcgcatcaa

SEQ ID NO: 29 - DNA, 30 bp, synthetic construct
  source 1..30: mol_type = other DNA
aagtacgttttgcggctgttggtttgcttg

SEQ ID NO: 30 - DNA, 30 bp, synthetic construct
  source 1..30: mol_type = other DNA
aatcattctttttgaaagcgggattccagg

SEQ ID NO: 31 - DNA, 30 bp, synthetic construct
  source 1..30: mol_type = other DNA
agcaagcatagcttgagaagcctgagaaag